European Patent Application EP 4 166 159 A1, published April 19, 2023. Title: PHARMACEUTICAL COMPOSITION OF ANTI-IL-17A ANTIBODIES AND USE THEREOF. Applicant: SHANGHAI JUNSHI BIOSCIENCES CO., LTD. SUZHOU JUNMENG BIOSCIENCES CO., LTD. SHANGHAI JUNSHI BIOTECHNOLOGY CO., LTD. The sequence listing filed with the application follows.

SEQUENCE LISTING (36 sequences)

SEQ ID NO: 1 - protein, 8 aa, Artificial Sequence
  HCDR1
GYIFTNYG

SEQ ID NO: 2 - protein, 8 aa, Artificial Sequence
  HCDR2
INDHTGEP

SEQ ID NO: 3 - protein, 10 aa, Artificial Sequence
  HCDR3
ANYGFGYFDY

SEQ ID NO: 4 - protein, 11 aa, Artificial Sequence
  LCDR1
QSLVHSNGNSY

SEQ ID NO: 5 - protein, 3 aa, Artificial Sequence
  LCDR2
KVS

SEQ ID NO: 6 - protein, 9 aa, Artificial Sequence
  LCDR3
SQSTHVPYT

SEQ ID NO: 7 - protein, 5 aa, Artificial Sequence
  HCDR1
SDYAW

SEQ ID NO: 8 - protein, 16 aa, Artificial Sequence
  HCDR2
FISYSGPTSYNPSLKS

SEQ ID NO: 9 - protein, 9 aa, Artificial Sequence
  HCDR3
GGDGDSFDY

SEQ ID NO: 10 - protein, 16 aa, Artificial Sequence
  LCDR1
RSSQSIVHSNGNTYLD

SEQ ID NO: 11 - protein, 7 aa, Artificial Sequence
  LCDR2
KVSNRFS

SEQ ID NO: 12 - protein, 8 aa, Artificial Sequence
  LCDR3
FQGSHFPT

SEQ ID NO: 13 - protein, 9 aa, Artificial Sequence
  HCDR1
GYSITSDYA

SEQ ID NO: 14 - protein, 7 aa, Artificial Sequence
  HCDR2
ISYSGPT

SEQ ID NO: 15 - protein, 11 aa, Artificial Sequence
  HCDR3
ARGGDGDSFDY

SEQ ID NO: 16 - protein, 11 aa, Artificial Sequence
  LCDR1
QSIVHSNGNTY

SEQ ID NO: 17 - protein, 3 aa, Artificial Sequence
  LCDR2
KVS

SEQ ID NO: 18 - protein, 8 aa, Artificial Sequence
  LCDR3
FQGSHFPT

SEQ ID NO: 19 - protein, 117 aa, Artificial Sequence
  VH
QVQLVQSGAEVKKPGASVKVSCKASGYIFTNYGMNWMRQAPGQGLEWMGWINDHTGEPTYADKFQGRVTFTLDTSISTAYMELSRLRSDDTAVYYCANYGFGYFDYWGQGTLVTVSS

SEQ ID NO: 20 - protein, 112 aa, Artificial Sequence
  VL
DVVMTQSPLSLPVTLGQPASISCRSSQSLVHSNGNSYLHWYLQKPGQSPQLLIYKVSNRFSGVPDRFSGSGSGTDFTLKISRVEAEDVGVYYCSQSTHVPYTFGQGTKLEIK

SEQ ID NO: 21 - protein, 117 aa, Artificial Sequence
  VH
QIQLVQSGAEVKKPGASVKISCKASGYIFTNYGMNWMRQAPGQGLEWMGWINDHTGEPTYADKFQGRVTFTLDTSASTAYMELSRLRSDDTAVYYCANYGFGYFDYWGQGTLVTVSS

SEQ ID NO: 22 - protein, 112 aa, Artificial Sequence
  VL
DVVMTQSPLSLPVTLGQPASISCRSSQSLVHSNGNSYLHWYLQKPGQSPQLLIYKVSNRFSGVPDRFSGSGSGTDFTLKISRVEAEDVGVYFCSQSTHVPYTFGQGTKLEIK

SEQ ID NO: 23 - protein, 118 aa, Artificial Sequence
  VH
QVQLQESGPGLVKPSETLSLTCTVTGYSISSDYAWSWIRQPPGKGLEWIGFISYSGPTSYNPSLKSRVTISRDTSKNQFSLKLSSVTAADTAVYYCARGGDGDSFDYWGQGTLVTVSS

SEQ ID NO: 24 - protein, 111 aa, Artificial Sequence
  VL
DVVMTQSPLSLPVTLGQPASISCRSSQSIVHSNGNTYLDWYLQKPGKSPKLLIYKVSNRFSGVPDRFSGSGSGTDFTLKISRVEAEDLGVYYCFQGSHFPTFGQGTKLEIK

SEQ ID NO: 25 - protein, 111 aa, Artificial Sequence
  VL
DVVMTQSPLSLPVTLGQPASISCRSSQSIVHSNGNTYLDWYLQKPGQSPKLLIYKVSNRFSGVPDRFSGSGSGTSFTLKISRVEAEDLGVYYCFQGSHFPTFGQGTKLEIK

SEQ ID NO: 26 - protein, 118 aa, Artificial Sequence
  VH
QVQLQESGPGLVKPSETLSLTCTVSGYSITSDYAWSWIRQPPGKGLEWIGFISYSGPTSYNPSLKSRVTISRDTSKNQFFLQLKSVTAADTAVYYCARGGDGDSFDYWGQGTTVTVSS

SEQ ID NO: 27 - protein, 111 aa, Artificial Sequence
  VL
DVVMTQTPLSLSVTPGQPASISCKSSQSIVHSNGNTYLDWYLQKPGQSPKLLIYKVSNRFSGVPDRFSGSGSGTDFTLKISRVEAEDVGVYYCFQGSHFPTFGGGTKVEIK

SEQ ID NO: 28 - protein, 444 aa, Artificial Sequence
  HC
QVQLVQSGAEVKKPGASVKVSCKASGYIFTNYGMNWMRQAPGQGLEWMGWINDHTGEPTYADKFQGRVTFTLDTSISTAYMELSRLRSDDTAVYYCANYGFGYFDYWGQGTLVTVSSASTKGPSVFPLAPCSRSTSESTAALGCLVKDYFPEPVTVSWNSGALTSGVHTFPAVLQSSGLYSLSSVVTVPSSSLGTKTYTCNVDHKPSNTKVDKRVESKYGPPCPPCPAPEFLGGPSVFLFPPKPKDTLMISRTPEVTCVVVDVSQEDPEVQFNWYVDGVEVHNAKTKPREEQFNSTYRVVSVLTVLHQDWLNGKEYKCKVSNKGLPSSIEKTISKAKGQPREPQVYTLPPSQEEMTKNQVSLTCLVKGFYPSDIAVEWESNGQPENNYKTTPPVLDSDGSFFLYSRLTVDKSRWQEGNVFSCSVMHEALHNHYTQKSLSLSLGK

SEQ ID NO: 29 - protein, 219 aa, Artificial Sequence
  LC
DVVMTQSPLSLPVTLGQPASISCRSSQSLVHSNGNSYLHWYLQKPGQSPQLLIYKVSNRFSGVPDRFSGSGSGTDFTLKISRVEAEDVGVYYCSQSTHVPYTFGQGTKLEIKRTVAAPSVFIFPPSDEQLKSGTASVVCLLNNFYPREAKVQWKVDNALQSGNSQESVTEQDSKDSTYSLSSTLTLSKADYEKHKVYACEVTHQGLSSPVTKSFNRGEC

SEQ ID NO: 30 - protein, 444 aa, Artificial Sequence
  HC
QIQLVQSGAEVKKPGASVKISCKASGYIFTNYGMNWMRQAPGQGLEWMGWINDHTGEPTYADKFQGRVTFTLDTSASTAYMELSRLRSDDTAVYYCANYGFGYFDYWGQGTLVTVSSASTKGPSVFPLAPCSRSTSESTAALGCLVKDYFPEPVTVSWNSGALTSGVHTFPAVLQSSGLYSLSSVVTVPSSSLGTKTYTCNVDHKPSNTKVDKRVESKYGPPCPPCPAPEFLGGPSVFLFPPKPKDTLMISRTPEVTCVVVDVSQEDPEVQFNWYVDGVEVHNAKTKPREEQFNSTYRVVSVLTVLHQDWLNGKEYKCKVSNKGLPSSIEKTISKAKGQPREPQVYTLPPSQEEMTKNQVSLTCLVKGFYPSDIAVEWESNGQPENNYKTTPPVLDSDGSFFLYSRLTVDKSRWQEGNVFSCSVMHEALHNHYTQKSLSLSLGK

SEQ ID NO: 31 - protein, 219 aa, Artificial Sequence
  LC
DVVMTQSPLSLPVTLGQPASISCRSSQSLVHSNGNSYLHWYLQKPGQSPQLLIYKVSNRFSGVPDRFSGSGSGTDFTLKISRVEAEDVGVYFCSQSTHVPYTFGQGTKLEIKRTVAAPSVFIFPPSDEQLKSGTASVVCLLNNFYPREAKVQWKVDNALQSGNSQESVTEQDSKDSTYSLSSTLTLSKADYEKHKVYACEVTHQGLSSPVTKSFNRGEC

SEQ ID NO: 32 - protein, 445 aa, Artificial Sequence
  HC
QVQLQESGPGLVKPSETLSLTCTVTGYSISSDYAWSWIRQPPGKGLEWIGFISYSGPTSYNPSLKSRVTISRDTSKNQFSLKLSSVTAADTAVYYCARGGDGDSFDYWGQGTLVTVSSASTKGPSVFPLAPCSRSTSESTAALGCLVKDYFPEPVTVSWNSGALTSGVHTFPAVLQSSGLYSLSSVVTVPSSSLGTKTYTCNVDHKPSNTKVDKRVESKYGPPCPPCPAPEFLGGPSVFLFPPKPKDTLMISRTPEVTCVVVDVSQEDPEVQFNWYVDGVEVHNAKTKPREEQFNSTYRVVSVLTVLHQDWLNGKEYKCKVSNKGLPSSIEKTISKAKGQPREPQVYTLPPSQEEMTKNQVSLTCLVKGFYPSDIAVEWESNGQPENNYKTTPPVLDSDGSFFLYSRLTVDKSRWQEGNVFSCSVMHEALHNHYTQKSLSLSLGK

SEQ ID NO: 33 - protein, 218 aa, Artificial Sequence
  LC
DVVMTQSPLSLPVTLGQPASISCRSSQSIVHSNGNTYLDWYLQKPGKSPKLLIYKVSNRFSGVPDRFSGSGSGTDFTLKISRVEAEDLGVYYCFQGSHFPTFGQGTKLEIKRTVAAPSVFIFPPSDEQLKSGTASVVCLLNNFYPREAKVQWKVDNALQSGNSQESVTEQDSKDSTYSLSSTLTLSKADYEKHKVYACEVTHQGLSSPVTKSFNRGEC

SEQ ID NO: 34 - protein, 218 aa, Artificial Sequence
  LC
DVVMTQSPLSLPVTLGQPASISCRSSQSIVHSNGNTYLDWYLQKPGQSPKLLIYKVSNRFSGVPDRFSGSGSGTSFTLKISRVEAEDLGVYYCFQGSHFPTFGQGTKLEIKRTVAAPSVFIFPPSDEQLKSGTASVVCLLNNFYPREAKVQWKVDNALQSGNSQESVTEQDSKDSTYSLSSTLTLSKADYEKHKVYACEVTHQGLSSPVTKSFNRGEC

SEQ ID NO: 35 - protein, 445 aa, Artificial Sequence
  HC
QVQLQESGPGLVKPSETLSLTCTVSGYSITSDYAWSWIRQPPGKGLEWIGFISYSGPTSYNPSLKSRVTISRDTSKNQFFLQLKSVTAADTAVYYCARGGDGDSFDYWGQGTTVTVSSASTKGPSVFPLAPCSRSTSESTAALGCLVKDYFPEPVTVSWNSGALTSGVHTFPAVLQSSGLYSLSSVVTVPSSSLGTKTYTCNVDHKPSNTKVDKRVESKYGPPCPPCPAPEFLGGPSVFLFPPKPKDTLMISRTPEVTCVVVDVSQEDPEVQFNWYVDGVEVHNAKTKPREEQFNSTYRVVSVLTVLHQDWLNGKEYKCKVSNKGLPSSIEKTISKAKGQPREPQVYTLPPSQEEMTKNQVSLTCLVKGFYPSDIAVEWESNGQPENNYKTTPPVLDSDGSFFLYSRLTVDKSRWQEGNVFSCSVMHEALHNHYTQKSLSLSLGK

SEQ ID NO: 36 - protein, 218 aa, Artificial Sequence
  LC
DVVMTQTPLSLSVTPGQPASISCKSSQSIVHSNGNTYLDWYLQKPGQSPKLLIYKVSNRFSGVPDRFSGSGSGTDFTLKISRVEAEDVGVYYCFQGSHFPTFGGGTKVEIKRTVAAPSVFIFPPSDEQLKSGTASVVCLLNNFYPREAKVQWKVDNALQSGNSQESVTEQDSKDSTYSLSSTLTLSKADYEKHKVYACEVTHQGLSSPVTKSFNRGEC